European Patent Application EP 4 238 572 A1, published September 6, 2023. Title: Bone formation composition and use thereof. Applicant: NAGASAKI UNIVERSITY MEGAKARYON CORPORATION. Application JP2020-180042. The sequence listing filed with the application follows.

SEQUENCE LISTING (10 sequences)

SEQ ID NO: 1 - DNA, 18 bp, Artificial Sequence
  Forward primer for TNF-alpha
aatggcgtggagctgaga

SEQ ID NO: 2 - DNA, 19 bp, Artificial Sequence
  Reverse primer for TNF-alpha
tagacctgcccagactcgg

SEQ ID NO: 3 - DNA, 20 bp, Artificial Sequence
  Forward primer for INF-gamma
ctgttactgccaggacccat

SEQ ID NO: 4 - DNA, 22 bp, Artificial Sequence
  Reverse primer for IFN-gamma
acactcttttggatgctctggt

SEQ ID NO: 5 - DNA, 20 bp, Artificial Sequence
  Forward primer for IL-1beta
cacagaccttccaggagaat

SEQ ID NO: 6 - DNA, 20 bp, Artificial Sequence
  Reverse primer for IL-1beta
ttcaacacgcaggacaggta

SEQ ID NO: 7 - DNA, 19 bp, Artificial Sequence
  Forward primer for IL-6
gtacatcctcgacggcatc

SEQ ID NO: 8 - DNA, 19 bp, Artificial Sequence
  Reverse primer for IL-6
agccactggttctgtgcct

SEQ ID NO: 9 - DNA, 21 bp, Artificial Sequence
  Forward primer for GAPDH
ggagtccactggcgtcttcac

SEQ ID NO: 10 - DNA, 24 bp, Artificial Sequence
  Reverse primer for GAPDH
gctgatgatcttgaggctgttgtc